European Patent Application EP 4 458 853 A1, published November 6, 2024. Title: DEVELOPMENT OF NOVEL UPAR SINGLE-DOMAIN ANTIBODY. Applicant: PERSONGEN BIOTHERAPEUTICS (SUZHOU) CO., LTD. The sequence listing filed with the application follows.

SEQUENCE LISTING (54 sequences)

SEQ ID NO: 1 - protein, 125 aa, synthetic construct
  source 1..125: note = 1-B4-hFC
QVQLVESGGGLVQPGGSLRLSCAASGFTLDYYAIGWFRQAPGKEREGVSCISSTGGSTNYADSVKGRFTISRDNAKNTVYLQMNSLKPEDTAVYYCAADTHYLTVCYDRLGFDYWGQGTQVTVSS

SEQ ID NO: 2 - protein, 122 aa, synthetic construct
  source 1..122: note = 1-F1-hFC
EVQLAESGGGLVQPGGSLRLSCAASGFTFSSYTMSWVRQAPGKGLEWVSAIDSDGGVTSYADSVKGRFTISRDNAKNTLYLQMNSLKPEDTAVYYCANGGYCSGYGCYPRLLSQGTLVTVSS

SEQ ID NO: 3 - protein, 126 aa, synthetic construct
  source 1..126: note = 1-F9-hFC
QSLLVESGGGLVQPGGSLRLSCAASGFSLDYYAIGWFRQAPGKEREEVSCISSGGGSTNYADSVKGRFTISRDNAKNTVYLQMNSLKPEDTAVYYCAAKRNFMLYLVQCPYEYDYWGQGTQVTVSS

SEQ ID NO: 4 - protein, 115 aa, synthetic construct
  source 1..115: note = 1-F10-hFC
QVQLVESGGGLVQPGGSLRLSCAASGSILSIRAVGWYRQAPGKQRELVALITSDGTTHYALSVKGRFTISRDNAKTTVYLQMNSLKPEDTAVYYCNREDYARRYWGQGTQVTVSS

SEQ ID NO: 5 - protein, 125 aa, synthetic construct
  source 1..125: note = 1-G1-hFC
QVQLVESGGGLVQPGGSLRLSCAASGNSLRRYAIGWFRQAPGKEREGVVCISTVGGSSYYVDSVKGRFTISEDNVKNTAYLQMNSLEPEDTAVYYCAAANRLYCPAYGSAGYDYWGQGTQVTVSS

SEQ ID NO: 6 - protein, 125 aa, synthetic construct
  source 1..125: note = 1-G2-hFC
QSQLAESGGGLVQPGGSLRLSCVASRFSLDAYAIAWFRQAPGKEREGVSCISSIGGRTNYADPVKGRFTISRDNAKNTAYLEMNSLQPEDTAVYYCAAVQRLFGPCLLSGGMDYWGKGTPVTVSS

SEQ ID NO: 7 - protein, 125 aa, synthetic construct; identical to SEQ ID NO: 6
  source 1..125: note = 1-H2-hFC

SEQ ID NO: 8 - protein, 127 aa, synthetic construct
  source 1..127: note = 1-H8-hFC
QRQLVESGGGLVQPGGSLRLSCAVSEFTLDYYAIGWFRQAPGKEREGVSCISSSGGSTVYADSVKGRFTISADNAKNTVYLQMNSLKPEDTAVYYCAAGSLLLFRLCVSRLYEYDYWGQGTQVTVSS

SEQ ID NO: 9 - protein, 117 aa, synthetic construct
  source 1..117: note = 3-E03-hFC
AVQLVDSGGGLVQAGGSLRLSCAASGIRLSSNAMAWYRQAPGKQRGLVALITSDGTTNYVDSVKGRFTISRDNAKNTVYLQMNSLKPEDTAVYYCKREPYLSTRGYWGQGTQVTVSS

SEQ ID NO: 10 - protein, 127 aa, synthetic construct
  source 1..127: note = 3-E04-hFC
QLRLVESGGGLVQPGGSLRLSCAASGFTLDYYDIGWFRQAPGKEREGVSCIGRISGDTDYAESVKGRFTASRDNAKNTVYLQMNSLKPEDTAVYYCAAERRFFGGGCRRSVDNMDSWGKGTLVTVSS

SEQ ID NO: 11 - protein, 117 aa, synthetic construct
  source 1..117: note = 3-E06-hFC
EVQLVESGGGLVQAGGSLTLSCVASASGSILRLNAMGWYRQAPAKQRELVALITRDGSTNYPDSVKGRFTISRDNAKNTVYLQMSSLSPEDTAVYYCYVQNHYSNYWGQGTQVTVSS

SEQ ID NO: 12 - protein, 119 aa, synthetic construct
  source 1..119: note = 3-E09-hFC
AVQLVDSGGGLVQPGGSLRLSCAASGFTFSSYAMGWARQVPGKGLEWVSIIYRDGNTYYTDSVKGRFTISRDNAKNTVYLQMNSLKPEDTAVYYCAPVETVAARRRDYWGQGTQVNVSS

SEQ ID NO: 13 - protein, 119 aa, synthetic construct; identical to SEQ ID NO: 12
  source 1..119: note = 3-E10-hFC

SEQ ID NO: 14 - protein, 124 aa, synthetic construct
  source 1..124: note = 3-G07-hFC
RLQLVESGGGLVQPGGSLRLSCAVSGKALDYYSIGWFRQAPRKQREGVSCISSSGGSTNYADSVKGRFTISRDNAKDTVYLQMNSLKPEDTADYYCAVVSTVLCGLGIYEYDYWGQGTLVTVSS

SEQ ID NO: 15 - protein, 127 aa, synthetic construct
  source 1..127: note = 3-H02-hFC
QLTLVESGGGLVQPGGSLRLSCAASEFTLDYYAIGWFRQAPGKEREGVSCISSSDGSTYYADSVKGRFTISRDNAKNTVYLQMNSLKPEDTAVYYCAIGGLLLLRLWERGNYEFDYWGQGTQVTVSS

SEQ ID NO: 16 - protein, 8 aa, synthetic construct
  source 1..8: note = CDR
GFTLDYYA

SEQ ID NO: 17 - protein, 8 aa, synthetic construct
  source 1..8: note = CDR
ISSTGGST

SEQ ID NO: 18 - protein, 21 aa, synthetic construct
  source 1..21: note = CDR
YYCAADTHYLTVCYDRLGFDY

SEQ ID NO: 19 - protein, 8 aa, synthetic construct
  source 1..8: note = CDR
GFTFSSYT

SEQ ID NO: 20 - protein, 8 aa, synthetic construct
  source 1..8: note = CDR
IDSDGGVT

SEQ ID NO: 21 - protein, 18 aa, synthetic construct
  source 1..18: note = CDR
YYCANGGYCSGYGCYPRL

SEQ ID NO: 22 - protein, 8 aa, synthetic construct
  source 1..8: note = CDR
GFSLDYYA

SEQ ID NO: 23 - protein, 8 aa, synthetic construct
  source 1..8: note = CDR
ISSGGGST

SEQ ID NO: 24 - protein, 22 aa, synthetic construct
  source 1..22: note = CDR
YYCAAKRNFMLYLVQCPYEYDY

SEQ ID NO: 25 - protein, 8 aa, synthetic construct
  source 1..8: note = CDR
GSILSIRA

SEQ ID NO: 26 - protein, 8 aa, synthetic construct
  source 1..8: note = CDR
LITSDGTT

SEQ ID NO: 27 - protein, 12 aa, synthetic construct
  source 1..12: note = CDR
YYCNREDYARRY

SEQ ID NO: 28 - protein, 8 aa, synthetic construct
  source 1..8: note = CDR
GNSLRRYA

SEQ ID NO: 29 - protein, 8 aa, synthetic construct
  source 1..8: note = CDR
ISTVGGSS

SEQ ID NO: 30 - protein, 20 aa, synthetic construct
  source 1..20: note = CDR
YYCAAANRLYCPAYGSAGYD

SEQ ID NO: 31 - protein, 8 aa, synthetic construct
  source 1..8: note = CDR
RFSLDAYA

SEQ ID NO: 32 - protein, 8 aa, synthetic construct
  source 1..8: note = CDR
ISSIGGRT

SEQ ID NO: 33 - protein, 21 aa, synthetic construct
  source 1..21: note = CDR
YYCAAVQRLFGPCLLSGGMDY

SEQ ID NO: 34 - protein, 8 aa, synthetic construct
  source 1..8: note = CDR
GSTLDYYA

SEQ ID NO: 35 - protein, 8 aa, synthetic construct
  source 1..8: note = CDR
ISSSGGRT

SEQ ID NO: 36 - protein, 23 aa, synthetic construct
  source 1..23: note = CDR
YNCAAGGDLSCYGTPTSIWQYDL

SEQ ID NO: 37 - protein, 8 aa, synthetic construct
  source 1..8: note = CDR
EFTLDYYA

SEQ ID NO: 38 - protein, 8 aa, synthetic construct
  source 1..8: note = CDR
ISSSGGST

SEQ ID NO: 39 - protein, 23 aa, synthetic construct
  source 1..23: note = CDR
YYCAAGSLLLFRLCVSRLYEYDY

SEQ ID NO: 40 - protein, 8 aa, synthetic construct
  source 1..8: note = CDR
GIRLSSNA

SEQ ID NO: 41 - protein, 14 aa, synthetic construct
  source 1..14: note = CDR
YYCKREPYLSTRGY

SEQ ID NO: 42 - protein, 8 aa, synthetic construct
  source 1..8: note = CDR
GFTLDYYD

SEQ ID NO: 43 - protein, 8 aa, synthetic construct
  source 1..8: note = CDR
IGRISGDT

SEQ ID NO: 44 - protein, 23 aa, synthetic construct
  source 1..23: note = CDR
YYCAAERRFFGGGCRRSVDNMDS

SEQ ID NO: 45 - protein, 10 aa, synthetic construct
  source 1..10: note = CDR
ASASGSILRL

SEQ ID NO: 46 - protein, 8 aa, synthetic construct
  source 1..8: note = CDR
LITRDGST

SEQ ID NO: 47 - protein, 12 aa, synthetic construct
  source 1..12: note = CDR
YYCYVQNHYSNY

SEQ ID NO: 48 - protein, 8 aa, synthetic construct
  source 1..8: note = CDR
GFTFSSYA

SEQ ID NO: 49 - protein, 8 aa, synthetic construct
  source 1..8: note = CDR
IIYRDGNT

SEQ ID NO: 50 - protein, 16 aa, synthetic construct
  source 1..16: note = CDR
YYCAPVETVAARRRDY

SEQ ID NO: 51 - protein, 8 aa, synthetic construct
  source 1..8: note = CDR
GKALDYYS

SEQ ID NO: 52 - protein, 20 aa, synthetic construct
  source 1..20: note = CDR
YYCAVVSTVLCGLGIYEYDY

SEQ ID NO: 53 - protein, 8 aa, synthetic construct
  source 1..8: note = CDR
ISSSDGST

SEQ ID NO: 54 - protein, 23 aa, synthetic construct
  source 1..23: note = CDR
YYCAIGGLLLLRLWERGNYEFDY